European Patent Application EP 4 215 549 A1, published July 26, 2023. Title: Anti-4-1BB-anti-PD-L1 bispecific antibody, and pharmaceutical composition and use thereof. Applicant: BIOTHEUS INC. The sequence listing filed with the application follows.

SEQUENCE LISTING (22 sequences)

SEQ ID NO: 1 - protein, 484 aa, Artificial Sequence
  peptide chain of bispecific antibody Bi-400
QVQLVESGGGVVQPGRSLRLSCAASGSTFSIVAMGWYRQAPGKQRELVASIITGDGDTNYADSVKGRFTISRDNSKNTMYLQMNSLKPEDTAVYYCYARTGYGSSWLMGHEYDYWGQGTQVTVSSTHTCPPCPAPEAAGGPSVFLFPPKPKDTLMISRTPEVTCVVVDVSHEDPEVKFNWYVDGVEVHNAKTKPREEQYNSTYRVVSVLTVLHQDWLNGKEYKCKVSNKALPAPIEKTISKAKGQPREPQVYTLPPSREEMTKNQVSLTCLVKGFYPSDIAVEWESNGQPENNYKTTPPVLDSDGSFFLYSKLTVDKSRWQQGNVFSCSVMHEALHNHYTQKSLSLSPGGGGGSGGGGSGGGGSGGGGSEVQLQESGGGLVQPGGSLRLSCAASGFTFSSYWMYWLRQAPGKGLEWVSSINSDSSSTYYRDSVKGRFTISRDNAKNTLYLQMNSLKSEDTAVYYCAKDPGGYAKGQGTQVTVSS

SEQ ID NO: 2 - protein, 125 aa, Artificial Sequence
  anti 4-1BB nanobody HZ-L-Yr-13&14-16-01
QVQLVESGGGVVQPGRSLRLSCAASGSTFSIVAMGWYRQAPGKQRELVASIITGDGDTNYADSVKGRFTISRDNSKNTMYLQMNSLKPEDTAVYYCYARTGYGSSWLMGHEYDYWGQGTQVTVSS

SEQ ID NO: 3 - protein, 224 aa, Artificial Sequence
  IgG1 Fc (LALA)
THTCPPCPAPEAAGGPSVFLFPPKPKDTLMISRTPEVTCVVVDVSHEDPEVKFNWYVDGVEVHNAKTKPREEQYNSTYRVVSVLTVLHQDWLNGKEYKCKVSNKALPAPIEKTISKAKGQPREPQVYTLPPSREEMTKNQVSLTCLVKGFYPSDIAVEWESNGQPENNYKTTPPVLDSDGSFFLYSKLTVDKSRWQQGNVFSCSVMHEALHNHYTQKSLSLSPG

SEQ ID NO: 4 - protein, 115 aa, Artificial Sequence
  anti PD-L1 nanobody C-Ye-18-5
EVQLQESGGGLVQPGGSLRLSCAASGFTFSSYWMYWLRQAPGKGLEWVSSINSDSSSTYYRDSVKGRFTISRDNAKNTLYLQMNSLKSEDTAVYYCAKDPGGYAKGQGTQVTVSS

SEQ ID NO: 5 - protein, 20 aa, Artificial Sequence
  (G4S)4 linker
GGGGSGGGGSGGGGSGGGGS

SEQ ID NO: 6 - protein, 484 aa, Artificial Sequence
  peptide chain of bispecific antibody Bi-088
EVQLQESGGGLVQPGGSLRLSCAASGFTFSSYWMYWLRQAPGKGLEWVSSINSDSSSTYYRDSVKGRFTISRDNAKNTLYLQMNSLKSEDTAVYYCAKDPGGYAKGQGTQVTVSSTHTCPPCPAPEAAGGPSVFLFPPKPKDTLMISRTPEVTCVVVDVSHEDPEVKFNWYVDGVEVHNAKTKPREEQYNSTYRVVSVLTVLHQDWLNGKEYKCKVSNKALPAPIEKTISKAKGQPREPQVYTLPPSREEMTKNQVSLTCLVKGFYPSDIAVEWESNGQPENNYKTTPPVLDSDGSFFLYSKLTVDKSRWQQGNVFSCSVMHEALHNHYTQKSLSLSPGGGGGSGGGGSGGGGSGGGGSQVQLVESGGGVVQPGRSLRLSCAASGSTFSIVAMGWYRQAPGKQRELVASIITGDGDTNYADSVKGRFTISRDNSKNTMYLQMNSLKPEDTAVYYCYARTGYGSSWLMGHEYDYWGQGTQVTVSS

SEQ ID NO: 7 - protein, 486 aa, Artificial Sequence
  peptide chain #1 bispecific antibody Bi-401-091 or Bi-061-091
EVQLQESGGGLVQPGGSLRLSCAASGFTFSSYWMYWLRQAPGKGLEWVSSINSDSSSTYYRDSVKGRFTISRDNAKNTLYLQMNSLKSEDTAVYYCAKDPGGYAKGQGTQVTVSSDKTHTCPPCPAPEAAGGPSVFLFPPKPKDTLMISRTPEVTCVVVDVSHEDPEVKFNWYVDGVEVHNAKTKPREEQYNSTYRVVSVLTVLHQDWLNGKEYKCKVSNKALPAPIEKTISKAKGQPREPQVCTLPPSRDELTKNQVSLSCAVKGFYPSDIAVEWESNGQPENNYKTTPPVLDSDGSFFLVSKLTVDKSRWQQGNVFSCSVMHEALHNHYTQKSLSLSPGGGGGSGGGGSGGGGSGGGGSQVQLVESGGGVVQPGRSLRLSCAASGSTFSIVAMGWYRQAPGKQRELVASIITGDGDTNYADSVKGRFTISRDNSKNTMYLQMNSLKPEDTAVYYCYARTGYGSSWLMGHEYDYWGQGTQVTVSS

SEQ ID NO: 8 - protein, 226 aa, Artificial Sequence
  IgG1 Fc (LALA) with a hole mutation
DKTHTCPPCPAPEAAGGPSVFLFPPKPKDTLMISRTPEVTCVVVDVSHEDPEVKFNWYVDGVEVHNAKTKPREEQYNSTYRVVSVLTVLHQDWLNGKEYKCKVSNKALPAPIEKTISKAKGQPREPQVCTLPPSRDELTKNQVSLSCAVKGFYPSDIAVEWESNGQPENNYKTTPPVLDSDGSFFLVSKLTVDKSRWQQGNVFSCSVMHEALHNHYTQKSLSLSPG

SEQ ID NO: 9 - protein, 226 aa, Artificial Sequence
  peptide chain #2 of bispecific antibody Bi-401-091
DKTHTCPPCPAPEAAGGPSVFLFPPKPKDTLMISRTPEVTCVVVDVSHEDPEVKFNWYVDGVEVHNAKTKPREEQYNSTYRVVSVLTVLHQDWLNGKEYKCKVSNKALPAPIEKTISKAKGQPREPQVYTLPPCRDELTKNQVSLWCLVKGFYPSDIAVEWESNGQPENNYKTTPPVLDSDGSFFLYSKLTVDKSRWQQGNVFSCSVMHEALHNHYTQKSLSLSPG

SEQ ID NO: 10 - protein, 341 aa, Artificial Sequence
  peptide chain #2 of bispecific antibody Bi-061-091
EVQLQESGGGLVQPGGSLRLSCAASGFTFSSYWMYWLRQAPGKGLEWVSSINSDSSSTYYRDSVKGRFTISRDNAKNTLYLQMNSLKSEDTAVYYCAKDPGGYAKGQGTQVTVSSDKTHTCPPCPAPEAAGGPSVFLFPPKPKDTLMISRTPEVTCVVVDVSHEDPEVKFNWYVDGVEVHNAKTKPREEQYNSTYRVVSVLTVLHQDWLNGKEYKCKVSNKALPAPIEKTISKAKGQPREPQVYTLPPCRDELTKNQVSLWCLVKGFYPSDIAVEWESNGQPENNYKTTPPVLDSDGSFFLYSKLTVDKSRWQQGNVFSCSVMHEALHNHYTQKSLSLSPG

SEQ ID NO: 11 - protein, 466 aa, Artificial Sequence
  peptide chain of control antobody INBRX-105-1B
EVQLLESGGGEVQPGGSLRLSCAASGGIFAIKPISWYRQAPGKQREWVSTTTSSGATNYAESVKGRFTISRDNAKNTLYLQMSSLRAEDTAVYYCNVFEYWGQGTLVTVKPGGSGGSEVQLLESGGGEVQPGGSLRLSCAASGFSFSINAMGWYRQAPGKRREFVAAIESGRNTVYAESVKGRFTISRDNAKNTVYLQMSSLRAEDTAVYYCGLLKGNRVVSPSVAYWGQGTLVTVKPGGGGDKTHTCPPCPAPGGPSVFLFPPKPKDTLMISRTPEVTCVVVDVSHEDPEVKFNWYVDGVEVHNAKTKPREEQYNSTYRVVSVLTVLHQDWLNGKEYKCKVSNKALPAPIEKTISKAKGQPREPQVYTLPPSRDELTKNQVSLTCLVKGFYPSDIAVEWESNGQPENNYKTTPPVLDSDGSFFLYSKLTVDKSRWQQGNVFSCSVMHEALHNHYTQKSLSLSPGK

SEQ ID NO: 12 - protein, 442 aa, Artificial Sequence
  heavy chain of Utomilumab
EVQLVQSGAEVKKPGESLRISCKGSGYSFSTYWISWVRQMPGKGLEWMGKIYPGDSYTNYSPSFQGQVTISADKSISTAYLQWSSLKASDTAMYYCARGYGIFDYWGQGTLVTVSSASTKGPSVFPLAPCSRSTSESTAALGCLVKDYFPEPVTVSWNSGALTSGVHTFPAVLQSSGLYSLSSVVTVPSSNFGTQTYTCNVDHKPSNTKVDKTVERKCCVECPPCPAPPVAGPSVFLFPPKPKDTLMISRTPEVTCVVVDVSHEDPEVQFNWYVDGVEVHNAKTKPREEQFNSTFRVVSVLTVVHQDWLNGKEYKCKVSNKGLPAPIEKTISKTKGQPREPQVYTLPPSREEMTKNQVSLTCLVKGFYPSDIAVEWESNGQPENNYKTTPPMLDSDGSFFLYSKLTVDKSRWQQGNVFSCSVMHEALHNHYTQKSLSLSPGK

SEQ ID NO: 13 - protein, 214 aa, Artificial Sequence
  light chain of Utomilumab
SYELTQPPSVSVSPGQTASITCSGDNIGDQYAHWYQQKPGQSPVLVIYQDKNRPSGIPERFSGSNSGNTATLTISGTQAMDEADYYCATYTGFGSLAVFGGGTKLTVLGQPKAAPSVTLFPPSSEELQANKATLVCLISDFYPGAVTVAWKADSSPVKAGVETTTPSKQSNNKYAASSYLSLTPEQWKSHRSYSCQVTHEGSTVEKTVAPTECS

SEQ ID NO: 14 - protein, 448 aa, Artificial Sequence
  heavy chain of urelumab
QVQLQQWGAGLLKPSETLSLTCAVYGGSFSGYYWSWIRQSPEKGLEWIGEINHGGYVTYNPSLESRVTISVDTSKNQFSLKLSSVTAADTAVYYCARDYGPGNYDWYFDLWGRGTLVTVSSASTKGPSVFPLAPCSRSTSESTAALGCLVKDYFPEPVTVSWNSGALTSGVHTFPAVLQSSGLYSLSSVVTVPSSSLGTKTYTCNVDHKPSNTKVDKRVESKYGPPCPPCPAPEFLGGPSVFLFPPKPKDTLMISRTPEVTCVVVDVSQEDPEVQFNWYVDGVEVHNAKTKPREEQFNSTYRVVSVLTVLHQDWLNGKEYKCKVSNKGLPSSIEKTISKAKGQPREPQVYTLPPSQEEMTKNQVSLTCLVKGFYPSDIAVEWESNGQPENNYKTTPPVLDSDGSFFLYSRLTVDKSRWQEGNVFSCSVMHEALHNHYTQKSLSLSLGK

SEQ ID NO: 15 - protein, 216 aa, Artificial Sequence
  light chain of urelumab
EIVLTQSPATLSLSPGERATLSCRASQSVSSYLAWYQQKPGQAPRLLIYDASNRATGIPARFSGSGSGTDFTLTISSLEPEDFAVYYCQQRSNWPPALTFCGGTKVEIKRTVAAPSVFIFPPSDEQLKSGTASVVCLLNNFYPREAKVQWKVDNALQSGNSQESVTEQDSKDSTYSLSSTLTLSKADYEKHKVYACEVTHQGLSSPVTKSFNRGEC

SEQ ID NO: 16 - protein, 9 aa, Artificial Sequence
  HZ-L-Yr-13&14-16-01 HCDR1
SGSTFSIVA

SEQ ID NO: 17 - protein, 9 aa, Artificial Sequence
  HZ-L-Yr-13&14-16-01 HCDR2
IITGDGDTN

SEQ ID NO: 18 - protein, 18 aa, Artificial Sequence
  HZ-L-Yr-13&14-16-01 HCDR3
YARTGYGSSWLMGHEYDY

SEQ ID NO: 19 - protein, 8 aa, Artificial Sequence
  C-Ye-18-5 HCDR1
GFTFSSYW

SEQ ID NO: 20 - protein, 8 aa, Artificial Sequence
  C-Ye-18-5 HCDR2
INSDSSST

SEQ ID NO: 21 - protein, 8 aa, Artificial Sequence
  C-Ye-18-5 HCDR3
AKDPGGYA

SEQ ID NO: 22 - protein, 21 aa, Artificial Sequence
  (G4S)4G linker
GGGGSGGGGSGGGGSGGGGSG